European Patent Application EP 4 166 666 A1, published April 19, 2023. Title: HIGH PURITY RNA COMPOSITIONS AND METHODS FOR PREPARATION THEREOF. Applicant: Moderna Therapeutics, Inc. Application Not Yet Assigned. The sequence listing filed with the application follows.

SEQUENCE LISTING (32 sequences)

SEQ ID NO: 1 - RNA, 12 nt, Artificial Sequence
  Synthetic Polynucleotide
cucuuauuuccc

SEQ ID NO: 2 - RNA, 49 nt, Artificial Sequence
  Synthetic Polynucleotide
  misc_feature (1)..(1): Modified by OH
  misc_feature (49)..(49): Modified by ppp
ggaaauaagagagaaaagacccuuuauucucucuuuucuucucauucuu

SEQ ID NO: 3 - RNA, 55 nt, Artificial Sequence
  Synthetic Polynucleotide
  misc_feature (1)..(1): Modified by OH
  misc_feature (55)..(55): Modified by ppp
gggaaauaagagagaaaagaagagucccuuuauucucucuuuucuucucauucuu

SEQ ID NO: 4 - RNA, 60 nt, Artificial Sequence
  Synthetic Polynucleotide
  misc_feature (1)..(1): Modified by OH
  misc_feature (60)..(60): Modified by ppp
gggaaauaagagagaaaagaagaguaagaacccuuuauucucucuuuucuucucauucuu

SEQ ID NO: 5 - RNA, 65 nt, Artificial Sequence
  Synthetic Polynucleotide
  misc_feature (1)..(1): Modified by OH
  misc_feature (65)..(65): Modified by ppp
gggaaauaagagagaaaagaagaguaagaagaaaucccuuuauucucucuuuucuucucauucuu

SEQ ID NO: 6 - RNA, 70 nt, Artificial Sequence
  Synthetic Polynucleotide
  misc_feature (1)..(1): Modified by OH
  misc_feature (70)..(70): Modified by ppp
gggaaauaagagagaaaagaagaguaagaagaaauauaagcccuuuauucucucuuuucuucucauucuu

SEQ ID NO: 7 - RNA, 12 nt, Artificial Sequence
  Synthetic Polynucleotide
  misc_feature (1)..(1): Modified by ppp
gggaaauaagag

SEQ ID NO: 8 - RNA, 12 nt, Artificial Sequence
  Synthetic Polynucleotide
  misc_feature (1)..(1): Modified by ppp
cucuuauuuccc

SEQ ID NO: 9 - RNA, 16 nt, Artificial Sequence
  Synthetic Polynucleotide
  misc_feature (1)..(1): Modified by ppp
  misc_feature (16)..(16): Modified by ppp
gggaaauacccuuuau

SEQ ID NO: 10 - RNA, 24 nt, Artificial Sequence
  Synthetic Polynucleotide
  misc_feature (1)..(1): Modified by ppp
  misc_feature (24)..(24): Modified by ppp
gggaaauaagagcccuuuauucuc

SEQ ID NO: 11 - RNA, 20 nt, Artificial Sequence
  Synthetic Polynucleotide
  misc_feature (1)..(1): Modified by ppp
  misc_feature (20)..(20): Modified by ppp
gggaaauacccuuuauucuc

SEQ ID NO: 12 - RNA, 20 nt, Artificial Sequence
  Synthetic Polynucleotide
  misc_feature (1)..(1): Modified by ppp
  misc_feature (20)..(20): Modified by ppp
gggaaauaagagcccuuuau

SEQ ID NO: 13 - RNA, 31 nt, Artificial Sequence
  Synthetic Polynucleotide
  misc_feature (1)..(1): Modified by ppp
  misc_feature (31)..(31): Modified by ppp
gggaaauaagagaaaagaagagucccuuuau

SEQ ID NO: 14 - RNA, 35 nt, Artificial Sequence
  Synthetic Polynucleotide
  misc_feature (1)..(1): Modified by ppp
  misc_feature (35)..(35): Modified by ppp
gggaaauaagagaaaagaagagucccuuuauucuc

SEQ ID NO: 15 - RNA, 40 nt, Artificial Sequence
  Synthetic Polynucleotide
  misc_feature (1)..(1): Modified by ppp
  misc_feature (40)..(40): Modified by ppp
gggaaauaagagagaaaagacccuuuauucucucuuuucu

SEQ ID NO: 16 - RNA, 41 nt, Artificial Sequence
  Synthetic Polynucleotide
  misc_feature (1)..(1): Modified by OH
  misc_feature (41)..(41): Modified by ppp
aaaaaaaaaaaaaaaaaaaaaaaaauuuuuuuuuuuuuuuu

SEQ ID NO: 17 - RNA, 45 nt, Artificial Sequence
  Synthetic Polynucleotide
  misc_feature (1)..(1): Modified by OH
  misc_feature (45)..(45): Modified by ppp
aaaaaaaaaaaaaaaaaaaaaaaaauuuuuuuuuuuuuuuuuuuu

SEQ ID NO: 18 - RNA, 49 nt, Artificial Sequence
  Synthetic Polynucleotide
  misc_feature (1)..(1): Modified by OH
  misc_feature (49)..(49): Modified by ppp
aaaaaaaaaaaaaaaaaaaaaaaaauuuuuuuuuuuuuuuuuuuuuuuu

SEQ ID NO: 19 - RNA, 43 nt, Artificial Sequence
  Synthetic Polynucleotide
  misc_feature (1)..(1): Modified by ppp
  misc_feature (43)..(43): Modified by ppp
gggaaauaagagaaaagaagagucccuuuauucucucuuuucu

SEQ ID NO: 20 - RNA, 40 nt, Artificial Sequence; identical to SEQ ID NO: 15
  Synthetic Polynucleotide
  misc_feature (1)..(1): Modified by ppp
  misc_feature (40)..(40): Modified by ppp

SEQ ID NO: 21 - RNA, 40 nt, Artificial Sequence; identical to SEQ ID NO: 15
  Synthetic Polynucleotide
  misc_feature (1)..(1): Modified by ppp
  misc_feature (40)..(40): Modified by OH

SEQ ID NO: 22 - RNA, 40 nt, Artificial Sequence; identical to SEQ ID NO: 15
  Synthetic Polynucleotide
  misc_feature (1)..(1): Modified by OH
  misc_feature (40)..(40): Modified by ppp

SEQ ID NO: 23 - RNA, 45 nt, Artificial Sequence
  Synthetic Polynucleotide
  misc_feature (1)..(1): Modified by OH
  misc_feature (45)..(45): Modified by ppp
gggaaauaagagagaaaagaagagucccuuuauucucucuuuucu

SEQ ID NO: 24 - RNA, 50 nt, Artificial Sequence
  Synthetic Polynucleotide
  misc_feature (1)..(1): Modified by OH
  misc_feature (50)..(50): Modified by ppp
gggaaauaagagagaaaagaagaguaagaacccuuuauucucucuuuucu

SEQ ID NO: 25 - RNA, 55 nt, Artificial Sequence
  Synthetic Polynucleotide
  misc_feature (1)..(1): Modified by OH
  misc_feature (55)..(55): Modified by ppp
gggaaauaagagagaaaagaagaguaagaagaaaucccuuuauucucucuuuucu

SEQ ID NO: 26 - RNA, 60 nt, Artificial Sequence
  Synthetic Polynucleotide
  misc_feature (1)..(1): Modified by OH
  misc_feature (60)..(60): Modified by ppp
gggaaauaagagagaaaagaagaguaagaagaaauauaagcccuuuauucucucuuuucu

SEQ ID NO: 27 - RNA, 67 nt, Artificial Sequence
  Synthetic Polynucleotide
  misc_feature (1)..(1): Modified by OH
  misc_feature (67)..(67): Modified by ppp
gggaaauaagagagaaaagaagaguaagaagaaauauaagagccacccccuuuauucucucuuuucu

SEQ ID NO: 28 - RNA, 26 nt, Artificial Sequence
  Synthetic Polynucleotide
gacucuucuuuucucucuuauuuccc

SEQ ID NO: 29 - RNA, 31 nt, Artificial Sequence
  Synthetic Polynucleotide
guucuuacucuucuuuucucucuuauuuccc

SEQ ID NO: 30 - RNA, 36 nt, Artificial Sequence
  Synthetic Polynucleotide
gauuucuucuuacucuucuuuucucucuuauuuccc

SEQ ID NO: 31 - RNA, 60 nt, Artificial Sequence
  Synthetic Polynucleotide
gggaaauaagagagaaaagaagaguaagaagaaauauaagagccaccaugggagugcacg

SEQ ID NO: 32 - RNA, 60 nt, Artificial Sequence
  Synthetic Polynucleotide
cgugcacucccaugguggcucuuauauuucuucuuacucuucuuuucucucuuauuuccc